European Patent Application EP 4 506 466 A1, published February 12, 2025. Title: Application of marker genes in detecting multipotent stem cell residues, detection method and kit. Applicant: IREGENE THERAPEUTICS, CO., LTD. The sequence listing filed with the application follows.

SEQUENCE LISTING (28 sequences)

SEQ ID NO: 1 - DNA, 1956 bp, Homo sapiens
agtttcccctggacgccttgctcctgcttctgctacgaccttctggggaaaacgaatttctcattttcttcttaaattgccattttcgctttaggagatgaatgttttcctttggctgttttggcaatgactctgaattaaagcgatgctaacgcctcttttccccctaattgttaaaagctatggactgcaggaagatggcccgcttctcttacagtgtgatttggatcatggccatttctaaagtctttgaactgggattagttgccgggctgggccatcaggaatttgctcgtccatctcggggatacctggccttcagagatgacagcatttggccccaggaggagcctgcaattcggcctcggtcttcccagcgtgtgccgcccatggggatacagcacagtaaggagctaaacagaacctgctgcctgaatgggggaacctgcatgctggggtccttttgtgcctgccctccctccttctacggacggaactgtgagcacgatgtgcgcaaagagaactgtgggtctgtgccccatgacacctggctgcccaagaagtgttccctgtgtaaatgctggcacggtcagctccgctgctttcctcaggcatttctacccggctgtgatggccttgtgatggatgagcacctcgtggcttccaggactccagaactaccaccgtctgcacgtactaccacttttatgctagttggcatctgcctttctatacaaagctactattaatcgacattgacctatttccagaaatacaattttagatatcatgcaaatttcatgaccagtaaaggctgctgctacaatgtcctaactgaaagatgatcatttgtagttgccttaaaataatgaatacatttccaaaatggtctctaacatttccttacagaactacttcttacttctttgccctgccctctcccaaaaaactacttcttttttcaaaagaaagtcagccatatctccattgtgcctaagtccagtgtttctttttttttttttttttgagacggagtctcactctgtcacccaggctggactgcaatgacgcgatcttggttcactgcaacctccgcatccggggttcaagccattctcctgcctcagcctcccaagtaactgggattacaggcatgtgtcaccatgcccagctaatttttttgtatttttagtagagatgggggtttcaccatattggccagtctggtctcgaactcctgaccttgtgatccactcgcctcagcctctcgaagtgctgagattacacacgtgagcaactgtgcaaggcctggtgtttcttgatacatgtaattctaccaaggtcttcttaatatgttcttttaaatgattgaattatatgttcagattattggagactaattctaatgtggaccttagaatacagttttgagtagagttgatcaaaatcaattaaaatagtctctttaaaaggaaagaaaacatctttaaggggaggaaccagagtgctgaaggaatggaagtccatctgcgtgtgtgcagggagactgggtaggaaagaggaagcaaatagaagagagaggttgaaaaacaaaatgggttacttgattggtgattaggtggtggtagagaagcaagtaaaaaggctaaatggaagggcaagtttccatcatctatagaaagctatataagacaagaactcccctttttttcccaaaggcattataaaaagaatgaagcctccttagaaaaaaaattatacctcaatgtccccaacaagattgcttaataaattgtgtttcctccaagctattcaattcttttaactgttgtagaagacaaaatgttcacaatatatttagttgtaaaccaagtgatcaaactacatattgtaaagcccatttttaaaatacattgtatatatgtgtatgcacagtaaaaatggaaactatattga

SEQ ID NO: 2 - DNA, 1998 bp, Homo sapiens
agctttttccctaaaggaaataccttggttcggtgtggtgactcattcctgtaatcccagtactttgggaggctgaagcaggcagattgcttgagcccaggagttcaagaccagcctgggaaaaatactgaaaccccgtctctacaaaaaatacaaaaattagccgggtgtggtcgtgcagcgcctgtaatcccagctactcaggaggtcaaggtgggagaatcacttgagcctgggagctcgaggctgtagtgagccgagattgcgccactgcattccagcctgggtgacagagcaagaccctgtctcaaaaaaaaaaaaaaaaaaaaaaaaggaaatacccaggattgctacaaagaaacaggcagctgccagaaatttgttggatttgaggagtccagagcgccgacccgctctgtctgcgtggacttatttccttggatcttcgtggactctgaagttgccaagtgtgtgtgcctgctccagaaaacaaaggaagccaccattttttctcattcacagtgcagggagatacctcagtagaagcatacagtccagtcttcaactagggacccctaccaggatgtccaaaaggctcagccctcagttacagcacaacatcacagaagatgcctattgtgaaacacacctggaaccaacacggctgttctgtgatgttgaccaaatcacactctgcagcaaatgcttccagtcccaggagcacaaacatcacatggtgtgtgggatacaagaggctgctgagaattacaggaagttattccaggaaatattgaacacatcgagggagaaacttgaagcagctaaaagcatattgactgatgagcaagaaagaatggcgatgattcaggaagaggaacaaaattttaaaaagatgattgagtctgagtatagtatgagactccggttgttgaatgaagagtgtgagcagaatctccagagacagcaggaatgcatatctgacttgaacctgagagaaacccttctgaatcaagcgatcaagcttgccaccgagctagaggagatgttccaggaaatgctacagagactgggccgtgtggggagagagaacatggagaaactgaaggagagtgaagccagggcttctgaacaggtccgcagcctcctaaagctcatcgtggagcttgagaaaaagtgtggggaaggcaccttggcattgctcaagaatgcaaaatactctttagaaaggagcaagtcactgctgcttgagcatctggagcccgctcatatcacagacctgagtttatgccacataagaggactcagcagcatgttcagagtactccagagacatttaacattggatcctgaaacagctcatccctgcctggcactatctgaggacctgagaactatgagattgagacatgggcagcaggatggggctggcaacccagaaagattggatttcagtgccatggtgctggctgcggagagcttcacctcagggaggcactactgggaggtggacgtggaaaaggcaaccaggtggcaagtgggcatataccacggctctgcagacgcgaagggcagcacggccagagcttccggagagaaagtcttgctcacggggtcggtgatggggaccgagtggactctctgggtcttcccccctctgaaaaggctcttcctggaaaagaagttggacacagttggcgttttccttgactgcgaacacgggcagatatcattctacaatgtgaccgagatgtccctcatttacaatttctcccattgcgccttccaaggagctctcaggcctgtgttttccctctgtatcccaaatggagacacaagtccagactccctcaccatcttacaacatggtccttcttgtgatgctactgttagcccttaatcttctgtgtgtaaaatccaagaccacgagacaccagaaagttggagaacaagactttgaaagaatttgtgtaaactaacccaataaaaagcgttccagga

SEQ ID NO: 3 - DNA, 24 bp, Artificial Sequence
  Chemically Synthesized
ggctgctgctacaatgtcctaact

SEQ ID NO: 4 - DNA, 24 bp, Artificial Sequence
  Chemically Synthesized
ggcacaatggagatatggctgact

SEQ ID NO: 5 - DNA, 23 bp, Artificial Sequence
  Chemically Synthesized
cacggctgttctgtgatgttgac

SEQ ID NO: 6 - DNA, 24 bp, Artificial Sequence
  Chemically Synthesized
tcctcttcctgaatcatcgccatt

SEQ ID NO: 7 - DNA, 20 bp, Artificial Sequence
  Chemically Synthesized
tcgtgcgtgacattaaggag

SEQ ID NO: 8 - DNA, 20 bp, Artificial Sequence
  Chemically Synthesized
ttgccaatggtgatgacctg

SEQ ID NO: 9 - DNA, 22 bp, Artificial Sequence
  Chemically Synthesized
gcctgaactgtagcagccagac

SEQ ID NO: 10 - DNA, 24 bp, Artificial Sequence
  Chemically Synthesized
cagccagtaagccaagaaggagtc

SEQ ID NO: 11 - DNA, 24 bp, Artificial Sequence
  Chemically Synthesized
gctggtggtacttccaatgaggta

SEQ ID NO: 12 - DNA, 24 bp, Artificial Sequence
  Chemically Synthesized
ccatctgggtaggtgacaaagagg

SEQ ID NO: 13 - DNA, 20 bp, Artificial Sequence
  Chemically Synthesized
tcgcacctgagcaagcacct

SEQ ID NO: 14 - DNA, 22 bp, Artificial Sequence
  Chemically Synthesized
ggagcacaggacatcggtcagt

SEQ ID NO: 15 - DNA, 23 bp, Artificial Sequence
  Chemically Synthesized
ggttcacagcctccagcatactc

SEQ ID NO: 16 - DNA, 23 bp, Artificial Sequence
  Chemically Synthesized
tgagcagccatcatcctccttgt

SEQ ID NO: 17 - DNA, 23 bp, Artificial Sequence
  Chemically Synthesized
tctgtcaacctgctggtcaatgc

SEQ ID NO: 18 - DNA, 22 bp, Artificial Sequence
  Chemically Synthesized
tgaaggagatggtgcggtcgtt

SEQ ID NO: 19 - DNA, 24 bp, Artificial sequence
  Chemically Synthesized
gcagtctcagtcacccgtgttatc

SEQ ID NO: 20 - DNA, 24 bp, Artificial Sequence
  Chemically Synthesized
gttgaccacaccattcctctccat

SEQ ID NO: 21 - DNA, 23 bp, Artificial Sequence
  Chemically Synthesized
ggtggactggaaggactggaaga

SEQ ID NO: 22 - DNA, 21 bp, Artificial Sequence
  Chemically Synthesized
ttgaagcggcaggcgaagatg

SEQ ID NO: 23 - DNA, 25 bp, Artificial Sequence
  Chemically Synthesized
atcttcaggagatatgcaaagcaga

SEQ ID NO: 24 - DNA, 20 bp, Artificial Sequence
  Chemically Synthesized
tgatctgctgcagtgtgggt

SEQ ID NO: 25 - DNA, 22 bp, Artificial Sequence
  Chemically Synthesized
acctcagctacaaacaggtgaa

SEQ ID NO: 26 - DNA, 20 bp, Artificial Sequence
  Chemically Synthesized
aaaggctggggtaggtaggt

SEQ ID NO: 27 - DNA, 22 bp, Artificial Sequence
  Chemically Synthesized
ttctgccatagtgtcctcttga

SEQ ID NO: 28 - DNA, 19 bp, Artificial Sequence
  Chemically Synthesized
agcctctcctagcctctgt